European Patent Application EP 4 481 046 A2, published December 25, 2024. Title: RNA AND NUCLEIC ACID CARRIER INCLUDING THE SAME. Applicant: LEMONEX INC. The sequence listing filed with the application follows.

SEQUENCE LISTING (49 sequences)

SEQ ID NO: 1 - RNA, 20 nt, synthetic construct
  misc_feature 1..20: note = siRNA
  source 1..20: mol_type = other RNA
cacacatatgccatggtgat

SEQ ID NO: 2 - RNA, 20 nt, synthetic construct
  misc_feature 1..20: note = siRNA
  source 1..20: mol_type = other RNA
cacacatatgccatggtgat

SEQ ID NO: 3 - RNA, 20 nt, synthetic construct
  misc_feature 1..20: note = siRNA
  source 1..20: mol_type = other RNA
tgacttatgagaacatggac

SEQ ID NO: 4 - RNA, 20 nt, synthetic construct
  misc_feature 1..20: note = siRNA
  source 1..20: mol_type = other RNA
gtccatgttctcataagtca

SEQ ID NO: 5 - RNA, 20 nt, synthetic construct
  misc_feature 1..20: note = siRNA
  source 1..20: mol_type = other RNA
tggagactgcagtaaaggat

SEQ ID NO: 6 - RNA, 20 nt, synthetic construct
  misc_feature 1..20: note = siRNA
  source 1..20: mol_type = other RNA
atcctttactgcagtctcca

SEQ ID NO: 7 - RNA, 20 nt, synthetic construct
  misc_feature 1..20: note = siRNA
  source 1..20: mol_type = other RNA
agctgcttctgcaatcaaag

SEQ ID NO: 8 - DNA, 20 bp, synthetic construct
  misc_feature 1..6: note = DNA
  misc_feature 7..20: note = RNA
  source 1..20: mol_type = other DNA; note = siRNA
ctttgattgcagaagcagct

SEQ ID NO: 9 - RNA, 19 nt, synthetic construct
  misc_feature 1..19: note = siRNA
  source 1..19: mol_type = other RNA
tgattcctgcaagccagca

SEQ ID NO: 10 - RNA, 19 nt, synthetic construct
  misc_feature 1..19: note = siRNA
  source 1..19: mol_type = other RNA
tgctggcttgcaggaatca

SEQ ID NO: 11 - RNA, 24 nt, synthetic construct
  misc_feature 1..24: note = siRNA
  source 1..24: mol_type = other RNA
agctgcttctgcaatcaaagtaat

SEQ ID NO: 12 - RNA, 24 nt, synthetic construct
  misc_feature 1..24: note = siRNA
  source 1..24: mol_type = other RNA
attactttgattgcagaagcagct

SEQ ID NO: 13 - DNA, 20 bp, synthetic construct
  misc_feature 1..20: note = CpG ODN
  source 1..20: mol_type = other DNA
gggggacgatcgtcgggggg

SEQ ID NO: 14 - DNA, 24 bp, synthetic construct
  misc_feature 1..24: note = CpG ODN
  source 1..24: mol_type = other DNA
tcgtcgttttgtcgttttgtcgtt

SEQ ID NO: 15 - DNA, 22 bp, synthetic construct
  misc_feature 1..22: note = CpG ODN
  source 1..22: mol_type = other DNA
tcgtcgttttcggcgcgcgccg

SEQ ID NO: 16 - RNA, 20 nt, synthetic construct
  misc_feature 1..20: note = siRNA
  source 1..20: mol_type = other RNA
tcaccatggcatatgtgtgg

SEQ ID NO: 17 - RNA, 20 nt, synthetic construct
  misc_feature 1..20: note = siRNA
  source 1..20: mol_type = other RNA
ccacacatatgccatggtga

SEQ ID NO: 18 - RNA, 19 nt, synthetic construct
  misc_feature 1..19: note = siRNA
  source 1..19: mol_type = other RNA
tctcatttcgtgatggaga

SEQ ID NO: 19 - RNA, 19 nt, synthetic construct
  misc_feature 1..19: note = siRNA
  source 1..19: mol_type = other RNA
tctccatcacgaaatgaga

SEQ ID NO: 20 - RNA, 19 nt, synthetic construct
  misc_feature 1..19: note = siRNA
  source 1..19: mol_type = other RNA
tctggctggaaaggcaacc

SEQ ID NO: 21 - RNA, 19 nt, synthetic construct
  misc_feature 1..19: note = siRNA
  source 1..19: mol_type = other RNA
ggttgcctttccagccaga

SEQ ID NO: 22 - RNA, 17 nt, synthetic construct
  misc_feature 1..17: note = siRNA
  source 1..17: mol_type = other RNA
ggtctggtgtatgaagg

SEQ ID NO: 23 - RNA, 20 nt, synthetic construct
  misc_feature 1..20: note = siRNA
  source 1..20: mol_type = other RNA
ccacacatatgccatggtga

SEQ ID NO: 24 - DNA, 21 bp, synthetic construct
  misc_feature 1..21: note = primer
  source 1..21: mol_type = other DNA
gatcctaataaccccctgact

SEQ ID NO: 25 - DNA, 18 bp, synthetic construct
  misc_feature 1..18: note = primer
  source 1..18: mol_type = other DNA
cagcatctgctccaccag

SEQ ID NO: 26 - DNA, 21 bp, synthetic construct
  misc_feature 1..21: note = primer
  source 1..21: mol_type = other DNA
tcactgccacccagaagactg

SEQ ID NO: 27 - DNA, 19 bp, synthetic construct
  misc_feature 1..19: note = primer
  source 1..19: mol_type = other DNA
ggatcaccttgcccacagc

SEQ ID NO: 28 - DNA, 23 bp, synthetic construct
  misc_feature 1..23: note = primer
  source 1..23: mol_type = other DNA
agctgcccgacgcatacagcccc

SEQ ID NO: 29 - DNA, 21 bp, synthetic construct
  misc_feature 1..21: note = primer
  source 1..21: mol_type = other DNA
accccagggccaggtgtgcca

SEQ ID NO: 30 - DNA, 20 bp, synthetic construct
  misc_feature 1..20: note = primer
  source 1..20: mol_type = other DNA
tggatttggacgcattggtc

SEQ ID NO: 31 - DNA, 21 bp, synthetic construct
  misc_feature 1..21: note = primer
  source 1..21: mol_type = other DNA
tttgcactggtacgtgttgat

SEQ ID NO: 32 - DNA, 1849 bp, Homo sapiens
  source 1..1849: mol_type = genomic DNA
actgaggggcaccagaggagcagactacaagaatggcacacgctatggaaaactcctggacaatcagtaaagagtaccatattgatgaagaagtgggctttgctctgccaaatccacaggaaaatctacctgatttttataatgactggatgttcattgctaaacatctgcctgatctcatagagtctggccagcttcgagaaagagttgagaagttaaacatgctcagcattgatcatctcacagaccacaagtcacagcgccttgcacgtctagttctgggatgcatcaccatggcatatgtgtggggcaaaggtcatggagatgtccgtaaggtcttgccaagaaatattgctgttccttactgccaactctccaagaaactggaactgcctcctattttggtttatgcagactgtgtcttggcaaactggaagaaaaaggatcctaataagcccctgacttatgagaacatggacgttttgttctcatttcgtgatggagactgcagtaaaggattcttcctggtctctctattggtggaaatagcagctgcttctgcaatcaaagtaattcctactgtattcaaggcaatgcaaatgcaagaacgggacactttgctaaaggcgctgttggaaatagcttcttgcttggagaaagcccttcaagtgtttcaccaaatccacgatcatgtgaacccaaaagcatttttcagtgttcttcgcatatatttgtctggctggaaaggcaacccccagctatcagacggtctggtgtatgaagggttctgggaagacccaaaggagtttgcagggggcagtgcaggccaaagcagcgtctttcagtgctttgacgtcctgctgggcatccagcagactgctggtggaggacatgctgctcagttcctccaggacatgagaagatatatgccaccagctcacaggaacttcctgtgctcattagagtcaaatccctcagtccgtgagtttgtcctttcaaaaggtgatgctggcctgcgggaagcttatgacgcctgtgtgaaagctctggtctccctgaggagctaccatctgcaaatcgtgactaagtacatcctgattcctgcaagccagcagccaaaggagaataagacctctgaagacccttcaaaactggaagccaaaggaactggaggcactgatttaatgaatttcctgaagactgtaagaagtacaactgagaaatcccttttgaaggaaggttaatgtaacccaacaagagcacattttatcatagcagagacatctgtatgcattcctgtcattacccattgtaacagagccacaaactaatactatgcaatgttttaccaataatgcaatacaaaagacctcaaaatacctgtgcatttcttgtaggaaaacaacaaaaggtaattatgtgtaattatactagaagttttgtaatctgtatcttatcattggaataaaatgacattcaataaataaaaatgcataagatatattctgtcggctgggcgcggtggctcacgcctgtaatcccagcactttgggaggccgaggcgggcggatcacaaggtcaggagatcgagaccatcttggctaacacggtgaaaccccgtctctactaaaaatacaaaaaattagccgggcgcggtggcgggcacctgtagtcccagctactcgggaggctgaggcaggagaatggcgtgaacctgggaggcggagcttgcagtgagccaagattgtgccactgcaatccggcctgggctaaagagcgggactccgtctcaaaaaaaaaaaaaaaaagatatattctgtcataataaataaaaatgcataagatataa

SEQ ID NO: 33 - DNA, 1473 bp, Canis familiaris
  source 1..1473: mol_type = genomic DNA
gtggtcattggctgtggcaacctttataataagtagaggctctgaaactctatcagaactaaggaccaaaagaggagactgcaagcatggaagatgatggaatacttcttatggaaagtcctcagagaatttttgaaaaataccatatagatgaagagatgggcttcgctttgccaaatccactggagaagctacctccgccttatgatgaatggatttccattgctaaaaatctgcctgaactgattaagaaaaatgaactacgtaaaaaagttgatgagttaaaaattctcagtattgatggccttagtggacacaagttgcagcgccttgcacgtctggctctggggtatatcaccatggcatatgtgtggaatcaaggtgatggagatgttcgaaaggtcttgccacagaatattgctattccttactgtgaactctctgagaagctgggtctgcctcctattctggtttatgcagactgtgtcttagcaaactggaagaaaaaggatcccaatgggcctatgacttatgagaacatggacattctcttctggtttcctggtggagactgcagtaaaggatttttcctggtttcactattggtggaattagcagctgcttctgcaatcaaagtaattcccaatttattaaaggcagttaaaaatcaggacgaggtcactttgaagaaggcactgcattatatagcttcttgtctgcaccgagcccataaagagtttgaagaagttcataaacatgtggacccaagcacgtttttcaaagttcttcgcatatacttgtctggttggaaaggcaactccaaactgccagagggtttgaagtatgaaggtttctgggaaaacccaaaagagtttgcaggaggcagtgcagcccaaagcagcatctttcaatgctttgacattctgctgggcatccagcagtgttctggtgaagaattcgctgctgaattcctccaggaaatgagaaactatatgcccccagctcaccgggactttcttctcttgttaaagtcaggcccctcagtccgggagtttgttcgttcaagagatgatgttgaactgaaggcagattataatgagtgtgtgaaagctatggtctccctgagaaaatatcacttgaagatagtagctaagtacattgtgattcctgcaagccagcagcccaagaataatcaagcatctgaagaatcatcggaacaaaaaaataaaggaactggaggcactaatgccatggatttcctgaagagtgtaagaactacaactgagaaattcctgctgatagatcattaatgtaactcaaacaagggcacattttgtcaagatgaagatgtctgtatatattagtgtcactgctcatgatatcagacccatgaattaatagtacacaacaatgttttttttttacaacaatgttttaatagtacttataaaagatttcaaaatatttttccaa

SEQ ID NO: 34 - RNA, 24 nt, Homo sapiens
  source 1..24: mol_type = unassigned RNA
agctgcttctgcaatcaaagtaat

SEQ ID NO: 35 - RNA, 24 nt, Homo sapiens
  source 1..24: mol_type = unassigned RNA
attactttgattgcagaagcagct

SEQ ID NO: 36 - RNA, 19 nt, Rattus norvegicus
  source 1..19: mol_type = unassigned RNA
gggcttcttcctcgtctct

SEQ ID NO: 37 - RNA, 19 nt, Rattus norvegicus
  source 1..19: mol_type = unassigned RNA
agagacgaggaagaagccc

SEQ ID NO: 38 - DNA, 20 bp, Homo sapiens
  source 1..20: mol_type = unassigned DNA
gggggacgatcgtcgggggg

SEQ ID NO: 39 - DNA, 20 bp, Rattus norvegicus
  source 1..20: mol_type = unassigned DNA
ggggtcaacgttgagggggg

SEQ ID NO: 40 - DNA, 20 bp, Homo sapiens
  source 1..20: mol_type = unassigned DNA
atcaccatggcatatgtgtg

SEQ ID NO: 41 - DNA, 20 bp, Homo sapiens
  source 1..20: mol_type = unassigned DNA
tgacttatgagaacatggac

SEQ ID NO: 42 - DNA, 20 bp, Homo sapiens
  source 1..20: mol_type = unassigned DNA
tggagactgcagtaaaggat

SEQ ID NO: 43 - DNA, 20 bp, Homo sapiens
  source 1..20: mol_type = unassigned DNA
agctgcttctgcaatcaaag

SEQ ID NO: 44 - DNA, 24 bp, Homo sapiens
  source 1..24: mol_type = unassigned DNA
agctgcttctgcaatcaaagtaat

SEQ ID NO: 45 - DNA, 19 bp, Homo sapiens
  source 1..19: mol_type = unassigned DNA
tgattcctgcaagccagca

SEQ ID NO: 46 - DNA, 20 bp, Homo sapiens
  source 1..20: mol_type = unassigned DNA
tcaccatggcatatgtgtgg

SEQ ID NO: 47 - DNA, 19 bp, Homo sapiens
  source 1..19: mol_type = unassigned DNA
tctcatttcgtgatggaga

SEQ ID NO: 48 - DNA, 19 bp, Homo sapiens
  source 1..19: mol_type = unassigned DNA
tctggctggaaaggcaacc

SEQ ID NO: 49 - DNA, 17 bp, Homo sapiens
  source 1..17: mol_type = unassigned DNA
ggtctggtgtatgaagg